European Patent Application EP 4 242 235 A1, published September 13, 2023. Title: Chimeric antibody receptor comprising anti mesothelin scFv and uses thereof. Applicant: Cellengene Inc. The sequence listing filed with the application follows.

SEQUENCE LISTING (15 sequences)

SEQ ID NO: 1 - protein, 5 aa, Artificial
  HCDR1 of MSLN3
DYAMS

SEQ ID NO: 2 - protein, 17 aa, Artificial
  HCDR2 of MSLN3
AISSSGGTTYYADSVKG

SEQ ID NO: 3 - protein, 12 aa, Artificial
  HCDR3 of MSLN3
EEEGEWREYFDV

SEQ ID NO: 4 - protein, 11 aa, Artificial
  LCDR1 of MSLN3
RASQSISSYLN

SEQ ID NO: 5 - protein, 7 aa, Artificial
  LCDR2 of MSLN3
ATSTLQS

SEQ ID NO: 6 - protein, 9 aa, Artificial
  LCDR3 of MSLN3
QQSYTFPYT

SEQ ID NO: 7 - protein, 121 aa, Artificial
  VH of MSLN3
EVQLVESGGGLVQPGGSLRLSCAASGFTFSDYAMSWVRQAPGKGLEWVSAISSSGGTTYYADSVKGRFTISRDNSKNTLYLQMNSLRAEDTAVYYCAKEEEGEWREYFDVWGQGTLVTVSS

SEQ ID NO: 8 - protein, 107 aa, Artificial
  VL of MSLN3
DIQMTQSPSSLSASVGDRVTITCRASQSISSYLNWYQQKPGKAPKLLIYATSTLQSGVPSRFSGSGSGTDFTLTISSLQPEDFATYYCQQSYTFPYTFGQGTKVEIK

SEQ ID NO: 9 - protein, 630 aa, Artificial
  mesothelin
MALPTARPLLGSCGTPALGSLLFLLFSLGWVQPSRTLAGETGQEAAPLDGVLANPPNISSLSPRQLLGFPCAEVSGLSTERVRELAVALAQKNVKLSTEQLRCLAHRLSEPPEDLDALPLDLLLFLNPDAFSGPQACTRFFSRITKANVDLLPRGAPERQRLLPAALACWGVRGSLLSEADVRALGGLACDLPGRFVAESAEVLLPRLVSCPGPLDQDQQEAARAALQGGGPPYGPPSTWSVSTMDALRGLLPVLGQPIIRSIPQGIVAAWRQRSSRDPSWRQPERTILRPRFRREVEKTACPSGKKAREIDESLIFYKKWELEACVDAALLATQMDRVNAIPFTYEQLDVLKHKLDELYPQGYPESVIQHLGYLFLKMSPEDIRKWNVTSLETLKALLEVNKGHEMSPQAPRRPLPQVATLIDRFVKGRGQLDKDTLDTLTAFYPGYLCSLSPEELSSVPPSSIWAVRPQDLDTCDPRQLDVLYPKARLAFQNMNGSEYFVKIQSFLGGAPTEDLKALSQQNVSMDLATFMKLRTDAVLPLTVAEVQKLLGPHVEGLKAEERHRPVRDWILRQRQDDLDTLGLGLQGGIPNGYLVLDLSMQEALSGTPCLLGPGPVLTVLALLLASTLA

SEQ ID NO: 10 - DNA, 63 bp, Artificial
  CD8 sequence
atggccttaccagtgaccgccttgctcctgccgctggccttgctgctccacgccgccaggccg

SEQ ID NO: 11 - DNA, 738 bp, Artificial
  MSLN3 scFv sequence
gaagtacagttggtcgaaagtggcggtggcctcgtgcaaccgggtggttcactgcgtctgagctgcgccgcctcgggttttactttctctgattatgcaatgtcttgggttcgtcaggcgccgggcaagggtctcgaatgggtttcagcaatctcttcttctggtggtactacttactatgccgattcagtgaagggtcgctttaccatttcccgtgacaactctaagaatactctgtatctgcagatgaactcgctgcgtgccgaagacacggccgtctattattgcgccaaagaagaagaaggtgaatggcgtgaatacttcgatgtttggggtcagggcactttagtgaccgtctcatcgggtggaggcggttcaggcggaggtggatccggcggtggcggatcggacattcaaatgacgcagagtccctcctcactgagtgctagcgtgggcgatcgtgtgacaattacttgtcgcgctagccagtctatctcttcttacctgaactggtatcagcagaaaccgggcaaggcgccaaaattgctgatttacgcaacttccactctgcagtctggtgtaccgtcccgtttctctggcagcggttctggtacggattttaccctgaccatctcaagcctccagcctgaagattttgccacctattattgtcagcaatcttacacttttccgtacacgttcgggcagggaactaaagtggaaattaaagccagcacc

SEQ ID NO: 12 - DNA, 135 bp, Artificial
  CD8 hinge sequence
accacgacgccagcgccgcgaccaccaacaccggcgcccaccatcgcgtcgcagcccctgtccctgcgcccagaggcgtgccggccagcggcggggggcgcagtgcacacgagggggctggacttcgcctgtgat

SEQ ID NO: 13 - DNA, 72 bp, Artificial
  CD8 TM sequence
atctacatctgggcgcccttggccgggacttgtggggtccttctcctgtcactggttatcaccctttactgc

SEQ ID NO: 14 - DNA, 126 bp, Artificial
  4-1BB sequence
aaacggggcagaaagaaactcctgtatatattcaaacaaccatttatgagaccagtacaaactactcaagaggaagatggctgtagctgccgatttccagaagaagaagaaggaggatgtgaactg

SEQ ID NO: 15 - DNA, 337 bp, Artificial
  CD3z sequence
agagtgaagttcagcaggagcgcagacgcccccgcgtacacagcagggccagaaccagctctataacgagctcaatctaggacgaagagaggagtacgatgttttggacaagagacgtggccgggaccctgagatggggggaaagccgagaaggaagaaccctcaggaaggcctgtacaatgaactgcagaaagataagatggcggaggcctacagtgagattgggatgaaaggcgagcgccggaggggcaaggggcacgatggcctttaccagggtctcagtacagccaccaaggacacctacgacgcccttcacatgcaggccctgccccctcgc